European Patent Specification EP 3 246 416 B1, published June 5, 2024. Title: Safe Sequencing System. Applicant: Vogelstein, Bert Kinzler, Kenneth W. Papadopoulos, Nickolas Kinde, Isaac. The sequence listing filed with the application follows.

SEQUENCE LISTING (81 sequences)

SEQ ID NO: 1 - DNA, 32 bp, Artificial Sequence
  Primers and adapters
gatcggaagagcggttcagcaggaatgccgag

SEQ ID NO: 2 - DNA, 33 bp, Artificial Sequence
  Primers and adapters
acactctttccctacacgacgctcttccgatct

SEQ ID NO: 3 - DNA, 62 bp, Artificial Sequence
  Primers and adapters
aatgatacggcgaccaccgagatctacacacactctttccctacacgacgctcttccgatct

SEQ ID NO: 4 - DNA, 57 bp, Artificial Sequence
  Primers and adapters
caagcagaagacggcatacgagatctcggcattcctgctgaaccgctcttccgatct

SEQ ID NO: 5 - DNA, 62 bp, Artificial Sequence; identical to SEQ ID NO: 3
  Primers and adapters

SEQ ID NO: 6 - DNA, 57 bp, Artificial Sequence; identical to SEQ ID NO: 4
  Primers and adapters

SEQ ID NO: 7 - DNA, 33 bp, Artificial Sequence; identical to SEQ ID NO: 2
  Primers and adapters

SEQ ID NO: 8 - DNA, 33 bp, Artificial Sequence
  Primers and adapters
ctcggcattcctgctgaaccgctcttccgatct

SEQ ID NO: 9 - DNA, 32 bp, Artificial Sequence; identical to SEQ ID NO: 1
  Primers and adapters

SEQ ID NO: 10 - DNA, 33 bp, Artificial Sequence; identical to SEQ ID NO: 2
  Primers and adapters

SEQ ID NO: 11 - DNA, 39 bp, Artificial Sequence
  Primers and adapters
cgtgatacactctttccctacacgacgctcttccgatct

SEQ ID NO: 12 - DNA, 39 bp, Artificial Sequence
  Primers and adapters
acatcgacactctttccctacacgacgctcttccgatct

SEQ ID NO: 13 - DNA, 39 bp, Artificial Sequence
  Primers and adapters
gcctaaacactctttccctacacgacgctcttccgatct

SEQ ID NO: 14 - DNA, 39 bp, Artificial Sequence
  Primers and adapters
tggtcaacactctttccctacacgacgctcttccgatct

SEQ ID NO: 15 - DNA, 39 bp, Artificial Sequence
  Primers and adapters
cactgtacactctttccctacacgacgctcttccgatct

SEQ ID NO: 16 - DNA, 39 bp, Artificial Sequence
  Primers and adapters
attggcacactctttccctacacgacgctcttccgatct

SEQ ID NO: 17 - DNA, 39 bp, Artificial Sequence
  Primers and adapters
gatctgacactctttccctacacgacgctcttccgatct

SEQ ID NO: 18 - DNA, 39 bp, Artificial Sequence
  Primers and adapters
tcaagtacactctttccctacacgacgctcttccgatct

SEQ ID NO: 19 - DNA, 39 bp, Artificial Sequence
  Primers and adapters
ctgatcacactctttccctacacgacgctcttccgatct

SEQ ID NO: 20 - DNA, 39 bp, Artificial Sequence
  Primers and adapters
aagctaacactctttccctacacgacgctcttccgatct

SEQ ID NO: 21 - DNA, 39 bp, Artificial Sequence
  Primers and adapters
gtagccacactctttccctacacgacgctcttccgatct

SEQ ID NO: 22 - DNA, 39 bp, Artificial Sequence
  Primers and adapters
tacaagacactctttccctacacgacgctcttccgatct

SEQ ID NO: 23 - DNA, 33 bp, Artificial Sequence; identical to SEQ ID NO: 8
  Primers and adapters

SEQ ID NO: 24 - DNA, 56 bp, Artificial Sequence
  Primers and adapters
aatgatacggcgaccaccgagatctacaccagcaggccttataataaaaataatga

SEQ ID NO: 25 - DNA, 51 bp, Artificial Sequence
  Primers and adapters
caagcagaagacggcatacgagattgactgaatataaacttgtggtagttg

SEQ ID NO: 26 - DNA, 33 bp, Artificial Sequence; identical to SEQ ID NO: 2
  Primers and adapters

SEQ ID NO: 27 - DNA, 33 bp, Artificial Sequence; identical to SEQ ID NO: 8
  Primers and adapters

SEQ ID NO: 28 - DNA, 29 bp, Artificial Sequence
  Primers and adapters
cggaagagcgtcgtgtagggaaagagtgt

SEQ ID NO: 29 - DNA, 29 bp, Artificial Sequence
  Primers and adapters
cggaagagcggttcagcaggaatgccgag

SEQ ID NO: 30 - DNA, 23 bp, Artificial Sequence
  Primers and adapters
ggttacaggctcatgatgtaacc

SEQ ID NO: 31 - DNA, 21 bp, Artificial Sequence
  Primers and adapters
gataccagcttggtaatggca

SEQ ID NO: 32 - DNA, 56 bp, Artificial Sequence
  Primers and adapters
  misc_feature (1)...(56): n = A,T,C or G
cgacgtaaaacgacggccagtnnnnnnnnnnnnggttacaggctcatgatgtaacc

SEQ ID NO: 33 - DNA, 46 bp, Artificial Sequence
  Primers and adapters
cacacaggaaacagctatgaccatggataccagcttggtaatggca

SEQ ID NO: 34 - DNA, 56 bp, Artificial Sequence
  Primers and adapters
aatgatacggcgaccaccgagatctacaccgtgatcgacgtaaaacgacggccagt

SEQ ID NO: 35 - DNA, 56 bp, Artificial Sequence
  Primers and adapters
aatgatacggcgaccaccgagatctacacacatcgcgacgtaaaacgacggccagt

SEQ ID NO: 36 - DNA, 56 bp, Artificial Sequence
  Primers and adapters
aatgatacggcgaccaccgagatctacacgcctaacgacgtaaaacgacggccagt

SEQ ID NO: 37 - DNA, 56 bp, Artificial Sequence
  Primers and adapters
aatgatacggcgaccaccgagatctacactggtcacgacgtaaaacgacggccagt

SEQ ID NO: 38 - DNA, 56 bp, Artificial Sequence
  Primers and adapters
aatgatacggcgaccaccgagatctacaccactgtcgacgtaaaacgacggccagt

SEQ ID NO: 39 - DNA, 56 bp, Artificial Sequence
  Primers and adapters
aatgatacggcgaccaccgagatctacacattggccgacgtaaaacgacggccagt

SEQ ID NO: 40 - DNA, 56 bp, Artificial Sequence
  Primers and adapters
aatgatacggcgaccaccgagatctacacgatctgcgacgtaaaacgacggccagt

SEQ ID NO: 41 - DNA, 56 bp, Artificial Sequence
  Primers and adapters
aatgatacggcgaccaccgagatctacactcaagtcgacgtaaaacgacggccagt

SEQ ID NO: 42 - DNA, 56 bp, Artificial Sequence
  Primers and adapters
aatgatacggcgaccaccgagatctacacctgatccgacgtaaaacgacggccagt

SEQ ID NO: 43 - DNA, 56 bp, Artificial Sequence
  Primers and adapters
aatgatacggcgaccaccgagatctacacaagctacgacgtaaaacgacggccagt

SEQ ID NO: 44 - DNA, 49 bp, Artificial Sequence
  Primers and adapters
caagcagaagacggcatacgagatcacacaggaaacagctatgaccatg

SEQ ID NO: 45 - DNA, 21 bp, Artificial Sequence
  Primers and adapters
cgacgtaaaacgacggccagt

SEQ ID NO: 46 - DNA, 21 bp, Artificial Sequence
  Primers and adapters
actggccgtcgttttacgtcg

SEQ ID NO: 47 - DNA, 58 bp, Artificial Sequence
  Primers and adapters
  misc_feature (1)...(58): n = A,T,C or G
cgacgtaaaacgacggccagtnnnnnnnnnnnnnngcagcaacagtcttacctggact

SEQ ID NO: 48 - DNA, 48 bp, Artificial Sequence
  Primers and adapters
cacacaggaaacagctatgaccatgtccacatcctcttcctcaggatt

SEQ ID NO: 49 - DNA, 50 bp, Artificial Sequence
  Primers and adapters
aatgatacggcgaccaccgagatctacaccgacgtaaaacgacggccagt

SEQ ID NO: 50 - DNA, 55 bp, Artificial Sequence
  Primers and adapters
caagcagaagacggcatacgagatatcacgcacacaggaaacagctatgaccatg

SEQ ID NO: 51 - DNA, 55 bp, Artificial Sequence
  Primers and adapters
caagcagaagacggcatacgagatcgatgtcacacaggaaacagctatgaccatg

SEQ ID NO: 52 - DNA, 55 bp, Artificial Sequence
  Primers and adapters
caagcagaagacggcatacgagattgaccacacacaggaaacagctatgaccatg

SEQ ID NO: 53 - DNA, 55 bp, Artificial Sequence
  Primers and adapters
caagcagaagacggcatacgagatgccaatcacacaggaaacagctatgaccatg

SEQ ID NO: 54 - DNA, 55 bp, Artificial Sequence
  Primers and adapters
caagcagaagacggcatacgagatcagatccacacaggaaacagctatgaccatg

SEQ ID NO: 55 - DNA, 55 bp, Artificial Sequence
  Primers and adapters
caagcagaagacggcatacgagatacttgacacacaggaaacagctatgaccatg

SEQ ID NO: 56 - DNA, 55 bp, Artificial Sequence
  Primers and adapters
caagcagaagacggcatacgagatgatcagcacacaggaaacagctatgaccatg

SEQ ID NO: 57 - DNA, 55 bp, Artificial Sequence
  Primers and adapters
caagcagaagacggcatacgagattagcttcacacaggaaacagctatgaccatg

SEQ ID NO: 58 - DNA, 55 bp, Artificial Sequence
  Primers and adapters
caagcagaagacggcatacgagatggctaccacacaggaaacagctatgaccatg

SEQ ID NO: 59 - DNA, 55 bp, Artificial Sequence
  Primers and adapters
caagcagaagacggcatacgagatcttgtacacacaggaaacagctatgaccatg

SEQ ID NO: 60 - DNA, 21 bp, Artificial Sequence
  Primers and adapters
cgacgtaaaacgacggccagt

SEQ ID NO: 61 - DNA, 25 bp, Artificial Sequence
  Primers and adapters
catggtcatagctgtttcctgtgtg

SEQ ID NO: 62 - DNA, 57 bp, Artificial Sequence
  Primers and adapters
  misc_feature (1)...(57): n = A,T,C or G
cgacgtaaaacgacggccagtnnnnnnnnnnnnnnttaccgagaaagctcacaagaa

SEQ ID NO: 63 - DNA, 45 bp, Artificial Sequence
  Primers and adapters
cacacaggaaacagctatgaccatgatgctaaggcgaggatgaaa

SEQ ID NO: 64 - DNA, 56 bp, Artificial Sequence; identical to SEQ ID NO: 35
  Primers and adapters

SEQ ID NO: 65 - DNA, 56 bp, Artificial Sequence; identical to SEQ ID NO: 36
  Primers and adapters

SEQ ID NO: 66 - DNA, 56 bp, Artificial Sequence; identical to SEQ ID NO: 37
  Primers and adapters

SEQ ID NO: 67 - DNA, 56 bp, Artificial Sequence; identical to SEQ ID NO: 39
  Primers and adapters

SEQ ID NO: 68 - DNA, 56 bp, Artificial Sequence; identical to SEQ ID NO: 40
  Primers and adapters

SEQ ID NO: 69 - DNA, 56 bp, Artificial Sequence; identical to SEQ ID NO: 41
  Primers and adapters

SEQ ID NO: 70 - DNA, 56 bp, Artificial Sequence; identical to SEQ ID NO: 42
  Primers and adapters

SEQ ID NO: 71 - DNA, 49 bp, Artificial Sequence; identical to SEQ ID NO: 44
  Primers and adapters

SEQ ID NO: 72 - DNA, 21 bp, Artificial Sequence
  Primers and adapters
cgacgtaaaacgacggccagt

SEQ ID NO: 73 - DNA, 21 bp, Artificial Sequence
  Primers and adapters
cctaattccccccatccttac

SEQ ID NO: 74 - DNA, 21 bp, Artificial Sequence
  Primers and adapters
actggccgtcgttttacgtcg

SEQ ID NO: 75 - DNA, 77 bp, Artificial Sequence
  Primers and adapters
ggttacaggctcatgatgtaacctctgtgtcttggtgtaactttaaaacatatttttgccattaccaagctggtatc

SEQ ID NO: 76 - DNA, 77 bp, Artificial Sequence
  Primers and adapters
ggttacaggctcatgatgtaacctctgtgtcttggtgsaactttaaaacatatttttgccattaccaagctggtatc

SEQ ID NO: 77 - DNA, 55 bp, Artificial Sequence
  Primers and adapters
  misc_feature (1)...(55): n = A,T,C or G
acactctttccctacacgacgctcnnnnnnnnnnnnggtgagtctgtgcaggcat

SEQ ID NO: 78 - DNA, 45 bp, Artificial Sequence
  Primers and adapters
ctcgagcactgtcctgactgagacgataccagcttggtaatggca

SEQ ID NO: 79 - DNA, 59 bp, Artificial Sequence
  Primers and adapters
aatgatacggcgaccaccgagatctacaccgtgatacactctttccctacacgacgctc

SEQ ID NO: 80 - DNA, 48 bp, Artificial Sequence
  Primers and adapters
caagcagaagacggcatacgagatctcgagcactgtcctgactgagac

SEQ ID NO: 81 - DNA, 24 bp, Artificial Sequence
  Primers and adapters
acactctttccctacacgacgctc